European Patent Application EP 4 239 066 A2, published September 6, 2023. Title: NEW SIALYLTRANSFERASES FOR IN VIVO SYNTHESIS OF 3'SL. Applicant: DSM IP Assets B.V. Application EP. The sequence listing filed with the application follows.

SEQUENCE LISTING (54 sequences)

SEQ ID NO: 1 - protein, 301 aa, Campylobacter lari
MVGGGNAVICGNGPSLKNIDYKRLPKEFDVFKCNQFYFEDRYFVGKNIKYAFFNPFVFFEQYYTSKKLIQNGEYIIENIVCSTFNLPLIDNENFIKLFPSYFCDALLGHEVLAKINDFFAFVKYNEIYENKRITSGIYMCAAAVALGYKNIYLTGIDFYDDKNNMYAFESKQHNILSLLPNFKNKDSVYEAHSKNFDLETLIFLKEKYNVNFYALNENSPISKYIDLAPIENSNFILKDKPSNYINDILIPNSKYKNTIYKVQNQDSKLKQNIYYKLFKDLFHLPSDIKHYLKEKYANKNR

SEQ ID NO: 2 - protein, 360 aa, Neisseria gonorrhoeae
MIFYTFDRVNQGERNAVSLLKDKLFNEEGKPVNLIFCYTILQMKVAERIMAQHPGERFYVVLMSENRNEKYDYYFNQIKDKAERAYFFYLPYGLNKSFNFIPTMAELKVKSMLLPKVKRIYLASLEKVSIAAFLSTYPDAEIKTFDDGTNNLIRESSYLGGEFAVNGAIKRNFARMMVGDWSIAKTRNASDEHYTIFKGLKNIMDDGRRKMTYLPLFDASELKAGDETGGTVRILLGSPDKEMKEISEKAAKNFNIQYVAPHPRQTYGLSGVTALNSPYVIEDYILREIKKNPHTRYEIYTFFSGAALTMKDFPNVHVYALKPASLPEDYWLKPVYALFRQADIPILAFDDKNQSHGKSK

SEQ ID NO: 3 - protein, 303 aa, Pasteurella oralis
MDEVERSRECKSVVVAGNGASLTQVDYSLLPVNYDVFRCNQFYFEDHYFLGKKIKAAFFTPGVLLEQYYTLYHLRKNNEYSVDKIILSSFNHPTVDLSKSENIKKLFIDVINGYEEYLSKLSDFDIYLRYKELYESQRITSGIYMCAVAIAMGYTDIYLTGIDFYESNSKSYAFEPKKTNIISLLPDFKNISSKFHYHNKDADLEALYFLQKNYSVNFYSISPGSLLYEHFPTSTKNISSQTNLIPVKKENYINDILLPPDFVYEKLGFVNSKKERLNANLIFRIIKDFIKLPSAIKHYLREK

SEQ ID NO: 4 - protein, 308 aa, Pasteurella
MNLIICCTPLQVLIAEKIIAKFPHTPFYGVMLSTVSNKKFDFYAKRLAQQCQGFFSMVQHKDRFNLLKEILYLKRTFSGKHFDQVFVANINDLQIQFLLSAIDFNLLNTFDDGTINIVPNSLFYQDDPATLQRKLINVLLGNKYSIQSLRALSHTHYTIYKGFKNIIERVKPIELVAADNSEKVTSAVINVLLGQPVFAEDERNIALAERVIKQFNIHYYLPHPREKYRLAQVNYIDTELIFEDYILQQCQTHKYCVYTYFSSAIINIMNKSDNIEVVALKIDTENPAYDACYDLFDELGVNVIDIRE

SEQ ID NO: 5 - protein, 342 aa, Neisseria meningitidis
MERNAVSLLKEKLFNEEGEPVNLIFCYTILQMKVAERIMAQHPGERFYVVLMSENRNEKYDYYFNQIKDKAERAYFFHLPYGLNKSFNFIPTMAELKVKSMLLPKVKRIYLASLEKVSIAAFLSTYPDAEIKTFDDGTGNLIQSSSYLGDEFSVNGTIKRNFARMMIGDWSIAKTRNASDEHYTIFKGLKNIMDDGRRKMTYLPLFDASELKTGDETGGTVRILLGSPDKEMKEISEKAAKNFKIQYVAPHPRQTYGLSGVTTLNSPYVIEDYILREIKKNPHTRYEIYTFFSGAALTMKDFPNVHVYALKPASLPEDYWLKPVYALFTQSGIPILTFDDKN

SEQ ID NO: 6 - protein, 272 aa, Pasteurella multocida
MDKFAEHEIPKAVIVAGNGESLSQIDYRLLPKNYDVFRCNQFYFEERYFLGNKIKAVFFTPGVFLEQYYTLYHLKRNNEYFVDNVILSSFNHPTVDLEKSQKIQALFIDVINGYEKYLSKLTAFDVYLRYKELYENQRITSGVYMCAVAIAMGYTDIYLTGIDFYQASEENYAFDNKKPNIIRLLPDFRKEKTLFSYHSKDIDLEALSFLQQHYHVNFYSISPMSPLSKHFPIPTVEDDCETTFVAPLKENYINDILLPPHFVYEKLGTIVS

SEQ ID NO: 7 - protein, 388 aa, Pasteurella multocida
MKTITLYLDPASLPALNQLMDFTQNNEDKTHPRIFGLSRFKIPDNIITQYQNIHFVELKDNRPTEALFTILDQYPGNIELNIHLNIAHSVQLIRPILAYRFKHLDRVSIQQLNLYDDGSMEYVDLEKEENKDISAEIKQAEKQLSHYLLTGKIKFDNPTIARYVWQSAFPVKYHFLSTDYFEKAEFLQPLKEYLAENYQKMDWTAYQQLTPEQQAFYLTLVGFNDEVKQSLEVQQAKFIFTGTTTWEGNTDVREYYAQQQLNLLNHFTQAEGDLFIGDHYKIYFKGHPRGGEINDYILNNAKNITNIPANISFEVLMMTGLLPDKVGGVASSLYFSLPKEKISHIIFTSNKQVKSKEDALNNPYVKVMRRLGIIDESQVIFWDSLKQL

SEQ ID NO: 8 - protein, 410 aa, Avibacterium avium
MKQFDVYLDYATLPSLNMMFDLVEKKDNQQIERIIGFERFNLSEDKLSAFPQGKISFSKVSLKDFTAFSDLLVNKIAQSDELVELFIHTNLDHSFYNLPNVLEKLSPIANKFTIKHLYLYDDGSMNYKDLYEHREQDIKKLLASSQNELAKKLASHSNNNELDSISRYTWHKFFPTDYILLRPDYLTIDEKMQPLKEFIGNNVSAMSWSRFEKLSPEQKTLFLKLVNVDENTLHKLKNNSEERTFIFTGTTTWEKDKDKRLANAKTQVKVLEDFLKPDGKFYLGNKIKVFFKGHPKGDEINEYILKQTGAENIPANIPFEVLMMTNSLPDYVGGIMSSMYFSLPATHINKVIFLDSDKVKNKNDAKAQTLSKLMLMLNVITPEQIAFEEIPETKKNSFFKQAFDTLRSKF

SEQ ID NO: 9 - protein, 312 aa, Mannheimiasp.
MNLIICCTPLQVLIAEKILEIHRNEQFFGVMLSTVKNAKFDFYQSRLAKKCQQFFAMQQHSERIQLLKEIIYLKSTFGGKKFNKVFLANINELEIQFLLSAINFNEINTFDDGIANIVQSGIFYKQECSGINRKLINTFLGNRYSLEKLKKLSKKHYTIYKGFPNIIENTVYIELINSTTLPDSELNNSEVVNILLGQPIFERDDEKNIILAEKVIRQFNIDRYFPHPREKYQISNVEYIKTNLILEDYLFQECSDKKCRVYTYFSSAVINILNKSPNIEVVALRVNVDNPTYIESYVLLENLGINIIDIRE

SEQ ID NO: 10 - protein, 300 aa, Campylobacter subantarcticus
MQGGGNAIICGNGPSLKDIDYKKLPRKYDVFRCNQFYFEEKYYLGKNIKYAFFNPFVFFEQYYTTKKLIEKKEYNIENIICSTFNLPTVDNENFIKNFNNYFCDAYLGHEILHNIKDFLAFIKYNELYENNRITSGIYMCAIAIALGYKNIYLCGIDFYNDKNNMYGFDNKKENLLKLNPEFLKKDSVYTKHSKEFDLKALEFLKEIYGVNFYSLNNNELSKYIPLAPNTNNNFVLIDKDKNYVNDILIPKEKDYCKLFKQEDGKIKLKENVYYKLFKDLFRLPSDIKHYLKEKYANKNR

SEQ ID NO: 11 - protein, 302 aa, Campylobacter coli
MQNVIIAGNGPSLQSINYQRLPKEYDIFRCNQFYFEDKYYLGKNIKAAFFNPYPFLQQYHTAKQLVFNNEYKIENIFCSTFNLPFIEKDNFINKFYDFFPDAKLGHKIIENLKEFYAYIKYNEIYLNKRITSGIYMCAIAIALGYKNIYLCGIDFYEGETIYPFKAMSKNIKKIFPWIKDFNPSNFHSKEYDIEILKLLESIYKVNIYALCDNSALANYFPLLVNTDNSFVLENKSDDCINDILLTNNTPGINFYKSQIQVNNTEILLLNFQNMISAKENEISNLNKILQDSYKTINTKENE

SEQ ID NO: 12 - protein, 259 aa, Campylobacter jejuni
MKKVIIAGNGPSLKEIDYSRLPNDFDVFRCNQFYFEDKYYLGKKCKAVFYNPILFFEQYYTLKHLIQNQEYETELIMCSNYNQAHLENENFVKTFYDYFPDAHLGYDFFKQLKDFNAYFKFHEIYFNQRITSGVYMCAVAIALGYKEIYLSGIDFYQNGSSYAFDTKQKNLLKLAPNFKNDNSHYIGHSKNTDIKALEFLEKTYKIKLYCLCPNSLLANFIELAPNLNSNFIIQEKNNYTKDILIPSSEAYGKFSKNIN

SEQ ID NO: 13 - DNA, 300 bp, synthetic construct
  misc_feature 1..300: note = Promoter sequence
  source 1..300: mol_type = other DNA
gcggcacgccttgcagattacggtttgccacacttttcatccttctcctggtgacataatccacatcaatcgaaaatgttaataaatttgttgcgcgaatgatctaacaaacatgcatcatgtacaatcagatggaataaatggcgcgataacgctcattttatgacgaggcacacacattttaagttcgatatttctcgtttttgctcgttaacgataagtttacagcatgcctacaagcatcgtggaggtccgtgactttcacgcatacaacaaacattaaccaaggaggaaacagct

SEQ ID NO: 14 - DNA, 300 bp, synthetic construct
  misc_feature 1..300: note = Promoter sequence
  source 1..300: mol_type = other DNA
gcggcacgccttgcagattacggtttgccacacttttcatccttctcctggtgacataatccacatcaatcgaaaatgttaataaatttgttgcgcgaatgatctaacaaacatgcatcatgtacaatcagatggaataaatggcgcgataacgctcattttatgacgaggcacacacattttaagttcgatatttctcgtttttgctcgttaacgataagtttacagcatgcctacaagcatcgtggaggtccgtgactttcacgcatacaacaaacattaaccaaattcgaaacagct

SEQ ID NO: 15 - DNA, 300 bp, synthetic construct
  misc_feature 1..300: note = Promoter sequence
  source 1..300: mol_type = other DNA
gcggcacgccttgcagattacggtttgccacacttttcatccttctcctggtgacataatccacatcaatcgaaaatgttaataaatttgttgcgcgaatgatctaacaaacatgcatcatgtacaatcagatggaataaatggcgcgataacgctcattttatgacgaggcacacacattttaagttcgatatttctcgtttttgctcgttaacgataagtttacagcatgcctacaagcatcgtggaggtccgtgactttcacgcatacaacaaacattaaccaagaacaaaacagct

SEQ ID NO: 16 - DNA, 300 bp, synthetic construct
  misc_feature 1..300: note = Promoter sequence
  source 1..300: mol_type = other DNA
gcggcacgccttgcagattacggtttgccacacttttcatccttctcctggtgacataatccacatcaatcgaaaatgttaataaatttgttgcgcgaatgatctaacaaacatgcatcatgtacaatcagatggaataaatggcgcgataacgctcattttatgacgaggcacacacattttaagttcgatatttctcgtttttgctcgttaacgataagtttacagcatgcctacaagcatcgtggaggtccgtgactttcacgcatacaacaaacattaaccaagagcaaaacagct

SEQ ID NO: 17 - DNA, 107 bp, Escherichia coli
  source 1..107: mol_type = other DNA
tgtgagttagctcactcattaggcaccccaggctttacactttatgcttccggctcgtatgttgtgtggaattgtgagcggataacaatttcacacaggaaacagct

SEQ ID NO: 18 - DNA, 141 bp, synthetic construct
  misc_feature 1..141: note = Promoter sequence
  source 1..141: mol_type = other DNA
tgtgagttagctcactcattaggcaccccaggctttacactttatgcttccggctcgtatgttgtgtggaatgcctacaagcatcgtggaggtccgtgactttcacgcatacaacaaacattaaccaaggaggaaacagct

SEQ ID NO: 19 - DNA, 203 bp, synthetic construct
  misc_feature 1..203: note = Promoter sequence
  source 1..203: mol_type = other DNA
tgcgtcgccattctgtcgcaacacgccagaatgcggcggcgatcactaactcaacaaatcaggcgatgtaaccgctttcaatctgtgagtgatttcacagtatcttaacaatgtgatagctatgattgcaccgtgcctacaagcatcgtggaggtccgtgactttcacgcatacaacaaacattaacaaaaaccggagatacc

SEQ ID NO: 20 - DNA, 203 bp, synthetic construct
  misc_feature 1..203: note = Promoter sequence
  source 1..203: mol_type = other DNA
tgcgtcgccattctgtcgcaacacgccagaatgcggcggcgatcactaactcaacaaatcaggcgatgtaaccgctttcaatctgtgagtgatttcacagtatcttaacaatgtgatagctatgattgcaccgtgcctacaagcatcgtggaggtccgtgactttcacgcatacaacaaacattaaccaaggaggaaacagct

SEQ ID NO: 21 - DNA, 203 bp, synthetic construct
  misc_feature 1..203: note = Promoter sequence
  source 1..203: mol_type = other DNA
tgcgtcgccattctgtcgcaacacgccagaatgcggcggcgatcactaactcaacaaatcaggcgatgtaaccgctttcaatctgtgagtgatttcacagtatcttaacaatgtgatagctatgattgcaccgtgcctacaagcatcgtggaggtccgtgactttcacgcatacaacaaacattaaccaactaggaaacagct

SEQ ID NO: 22 - DNA, 203 bp, synthetic construct
  misc_feature 1..203: note = Promoter sequence
  source 1..203: mol_type = other DNA
tgcgtcgccattctgtcgcaacacgccagaatgcggcggcgatcactaactcaacaaatcaggcgatgtaaccgctttcaatctgtgagtgatttcacagtatcttaacaatgtgatagctatgattgcaccgtgcctacaagcatcgtggaggtccgtgactttcacgcatacaacaaacattaaccaagagaaaaacagct

SEQ ID NO: 23 - DNA, 906 bp, Campylobacter lari
  source 1..906: mol_type = other DNA
atggttggtggtggtaatgcagttatttgtggtaatggtccgagcctgaaaaacatcgattataaacgtctgccgaaagaattcgacgtgtttaaatgcaaccagttctatttcgaggatcgctattttgtgggcaagaacatcaaatatgcctttttcaatccgttcgtgttcttcgagcagtattataccagcaaaaagctgattcagaacggcgaatatatcatcgaaaatattgtgtgcagcacctttaatctgccgctgattgataacgagaacttcattaaactgttcccgagctatttttgtgatgcactgctgggtcatgaagtgctggccaaaatcaatgatttctttgccttcgtgaagtacaacgagatctatgaaaataaacgtatcaccagcggcatctatatgtgtgccgcagcagttgcactgggctataaaaacatttatctgaccggcatcgatttctacgacgacaaaaataacatgtatgccttcgaaagcaagcagcataatattctgagcctgctgccgaacttcaaaaacaaagatagcgtttatgaagcccacagcaaaaactttgatctggaaaccctgatctttctgaaagaaaaatacaacgtgaacttttatgccctgaatgaaaatagcccgatcagcaaatatatcgatctggcaccgattgaaaactccaactttatcctgaaagataaaccgagcaactacatcaacgatattctgattccgaacagcaagtacaagaacaccatctataaagtgcagaaccaggacagcaaactgaaacagaacatctactacaaactgttcaaggacctgtttcatctgccgagcgatattaaacattatcttaaagagaaatacgccaacaaaaatcgctaa

SEQ ID NO: 24 - DNA, 1080 bp, Neisseria gonorrhoeae
  source 1..1080: mol_type = other DNA
atgatcttctatacctttgatcgcgtgaatcagggtgaacgtaatgcagttagcctgctgaaagataaactgtttaacgaagaaggcaaaccggtcaatctgatcttttgttataccatcctgcagatgaaagtggccgaacgtattatggcacagcatccgggtgaacgcttttatgttgttctgatgagcgaaaaccgcaacgagaaatatgattactactttaaccagatcaaggacaaagcagaacgtgcctatttcttttatctgccgtatggtctgaacaaaagctttaactttattccgaccatggccgagctgaaagttaaaagcatgctgctgccgaaagtgaaacgtatttatctggcaagcctggaaaaagttagcattgcagcatttctgagcacctatccggatgcagaaatcaaaacctttgatgatggcaccaataacctgattcgtgaaagcagctatttaggtggtgaatttgcagttaatggtgcgatcaaacgtaattttgcacgtatgatggttggcgattggagcattgcaaaaacccgtaatgcatccgatgaacactataccatctttaaaggcctgaagaacattatggatgatggtcgtcgtaaaatgacctatctgccgctgtttgatgcaagcgaactgaaagccggtgatgaaaccggtggcaccgttcgtattctgctgggtagtccggataaagaaatgaaagaaattagcgagaaagcagccaaaaacttcaacattcagtatgttgcaccgcatccgcgtcagacctatggtctgtcaggtgttaccgcactgaatagcccgtatgtgattgaagattatattctgcgcgagatcaaaaagaatccgcatacacgttatgagatctacacctttttcagcggtgcagcactgaccatgaaagattttccgaatgttcatgtgtatgcactgaaaccggcaagtctgccggaagattattggctgaaacctgtttatgcactgtttcgtcaggcagatattccgattctggcattcgatgataaaaatcagagccacggtaaaagcaaa

SEQ ID NO: 25 - DNA, 912 bp, Pasteurella oralis
  source 1..912: mol_type = other DNA
atggatgaagttgaacgtagccgtgaatgtaaaagcgttgttgttgcaggtaatggtgcaagtctgacccaggttgattatagcctgctgccggttaattatgatgtgtttcgttgcaaccagttctatttcgaggatcattattttctgggcaaaaagatcaaagcagccttttttacaccgggtgttctgctggaacagtattacaccctgtatcatctgcgcaaaaacaacgaatatagcgtggataaaatcatcctgagcagctttaatcatccgaccgttgatctgagcaaaagcgagaatatcaaaaagctgttcatcgatgtgatcaacggctatgaagaatacctgagcaaactgagcgatttcgatatttatctgcgctacaaagaactgtatgaaagccagcgtattaccagcggcatttatatgtgtgcagttgcaattgccatgggctataccgatatctatctgaccggtatcgatttctatgagagcaacagcaaaagctatgcctttgaaccgaaaaagaccaacattattagtctgctgcccgactttaaaaacatcagcagcaaatttcactaccacaacaaagatgcagatctggaagcactgtattttctgcaaaaaaactacagcgtgaacttttacagcattagtccgggttcactgctgtatgaacattttccgaccagcaccaaaaacattagctcacagaccaatctgattccggtgaagaaagagaactatatcaacgatattctgctgcctccggatttcgtttatgaaaaactgggttttgtgaatagcaaaaaagaacgcctgaatgccaacctgattttccgcattatcaaagactttatcaaactgccgagcgccatcaaacattatctgcgtgaaaaataa

SEQ ID NO: 26 - DNA, 1029 bp, Neisseria meningitidis
  source 1..1029: mol_type = other DNA
atggaacgtaacgccgtgagcctgctgaaagaaaaactgtttaacgaagaaggtgaaccggtcaatctgatcttctgctataccattctgcagatgaaagtggcagaacgtattatggctcaacatccgggcgaacgcttttatgtggttctgatgagtgaaaaccgtaacgaaaaatacgattactacttcaaccagatcaaagacaaagcagaacgcgcttatttctttcacctgccgtacggtctgaacaaatcgtttaatttcattccgacgatggcggaactgaaagttaaaagcatgctgctgccgaaagtcaaacgtatctatctggcatccctggaaaaagtgtcaattgcggcctttctgtccacctacccggatgctgaaatcaaaaccttcgatgacggcacgggtaacctgattcaaagctctagttatctgggcgatgaattttctgttaacggtacgatcaaacgtaatttcgcccgcatgatgatcggcgattggtctattgcgaaaacccgcaacgccagtgacgaacattacacgatcttcaaaggcctgaaaaacatcatggatgacggtcgtcgcaaaatgacctacctgccgctgttcgatgccagcgaactgaaaacgggcgacgaaaccggcggtacggttcgtattctgctgggttccccggataaagaaatgaaagaaatctcagaaaaagcagctaaaaacttcaaaatccagtatgtcgcaccgcacccgcgccaaacctacggtctgtcgggtgtgaccacgctgaacagcccgtatgttattgaagattacatcctgcgtgaaattaagaaaaacccgcatacccgctatgaaatctacacgtttttctctggtgcggccctgaccatgaaagattttccgaatgtccacgtgtatgcgctgaaaccggccagtctgccggaagactactggctgaaaccggtgtacgctctgttcacgcaatccggcatcccgattctgacctttgacgataaaaactaa

SEQ ID NO: 27 - DNA, 927 bp, Pasteurella
  source 1..927: mol_type = other DNA
atgaacctgattatttgttgtacaccgctgcaggttctgattgccgaaaagattattgcaaaatttccgcacacaccgttttatggtgttatgctgagcaccgttagcaacaaaaagtttgatttttatgccaaacgtctggcacagcagtgtcagggtttctttagcatggttcagcataaagatcgcttcaacctgctgaaagaaattctgtatctgaaacgtacctttagcggcaaacattttgatcaggtttttgtggccaacatcaatgacctgcagattcagtttctgctgagcgccattgattttaatctgctgaatacctttgatgatggcaccattaacattgttccgaacagcctgttttatcaggatgatccggcaacactgcagcgtaaactgattaatgttctgctgggtaacaaatacagcattcagagcctgcgtgcactgagtcatacccattataccatctataaaggcttcaaaaacatcatcgaacgcgtgaaaccgattgaactggttgcagcagataattcagaaaaagttaccagcgcagttattaacgtgctgctgggccagccggtttttgcagaagatgaacgtaatattgcactggccgaacgtgttatcaaacagtttaacatccattactatctgccgcatccgcgtgaaaaatatcgtctggcccaggttaactatattgataccgaactgatcttcgaggattatattctgcagcagtgccagacacacaaatattgcgtttatacctattttagcagcgcgatcatcaacatcatgaacaaaagcgataacattgaagtggtggccctgaaaattgatacagaaaatccggcatatgatgcctgctatgacctgtttgatgaactgggtgttaacgtgattgatatccgcgaataa

SEQ ID NO: 28 - DNA, 819 bp, Pasteurella multocida
  source 1..819: mol_type = other DNA
atggataaatttgccgaacatgaaattccgaaagccgttattgttgcaggtaatggtgaaagcctgagccagattgattatcgtctgctgccgaaaaactatgatgtgtttcgttgcaaccagttctatttcgaagaacgctattttctgggcaacaaaatcaaagccgtgttttttacaccgggtgtttttctggaacagtattacaccctgtatcatctgaaacgcaacaacgaatatttcgtggataatgtgattctgagcagctttaatcatccgaccgttgatctggaaaaaagccagaaaattcaggccctgtttatcgatgtgattaacggctatgaaaagtacctgagcaaactgaccgcatttgatgtttatctgcgctataaagaactgtatgaaaaccagcgtattaccagcggtgtttatatgtgtgcagttgcaattgccatgggctataccgatatttatctgaccggtatcgatttttatcaggccagcgaagaaaactatgccttcgataacaaaaagccgaacattattcgcctgctgcctgattttcgtaaagaaaaaaccctgtttagctaccacagcaaagatatcgatctggaagcactgagctttctgcagcagcattatcatgttaacttctatagcattagcccgatgagtccgctgagtaaacattttccgattccgaccgtggaagatgattgtgaaaccacctttgttgcaccgctgaaagagaactatattaacgatattctgctgcctccgcacttcgtttatgaaaaactgggcaccattgtgagctaa

SEQ ID NO: 29 - DNA, 1167 bp, Pasteurella multocida
  source 1..1167: mol_type = other DNA
atgaaaaccattacgctgtatttagatccggcaagcctgcctgcactgaaccagctgatggattttacccagaataacgaggataaaacccatccgcgtatctttggtctgagccgctttaaaatcccggataacattattacccagtaccagaacatccacttcgtggaactgaaagataatcgtccgaccgaagcactgtttaccattctggatcagtatccgggtaatatcgaactgaacatccatctgaatattgcccatagcgttcagctgattcgtccgattctggcatatcgttttaaacatctggatcgtgttagcattcagcagctgaacctgtatgatgatggtagcatggaatatgtggatctggaaaaagaagagaacaaagatatcagcgcagaaatcaaacaggcagaaaaacagctgagccattatctgctgaccggcaaaattaagtttgataatccgaccattgcgcgttatgtttggcagagcgcatttccggttaaatatcattttctgagcaccgactatttcgagaaagcagaatttctgcagccgctgaaagaatatctggcagaaaattaccagaaaatggattggaccgcatatcagcaactgacaccggaacagcaggcattttatctgaccctggttggttttaacgatgaagttaaacagagcctggaagttcagcaggccaaatttatctttaccggcaccaccacctgggaaggtaataccgatgttcgtgaatattatgcacagcaacagctgaatctgctgaatcattttacacaggccgaaggtgacctgtttattggtgatcattacaaaatctatttcaaaggtcatccgcgtggtggcgaaattaatgattatattctgaacaacgccaaaaacatcaccaacattccggcaaacattagctttgaagttctgatgatgaccggtctgctgccggataaagttggtggtgttgcaagcagcctgtattttagcctgccgaaagaaaaaatcagccacatcattttcaccagcaacaaacaggtgaaaagcaaagaagatgcactgaataacccgtacgttaaagttatgcgtcgtctgggtattattgatgaaagccaggttatcttttgggacagcctgaaacagctgtaa

SEQ ID NO: 30 - DNA, 1233 bp, Avibacterium avium
  source 1..1233: mol_type = other DNA
atgaaacagttcgatgtgtatctggattatgcaaccctgccgagcctgaatatgatgtttgatctggttgagaaaaaggacaaccagcagattgaacgcattattggttttgaacgctttaacctgagcgaggataaactgagcgcatttccgcagggtaaaattagctttagcaaagtgagcctgaaagattttaccgcatttagcgacctgctggttaacaaaattgcacagagtgatgaactggtggaactgtttattcataccaatctggatcacagcttttacaatctgccgaatgttctggaaaaactgagcccgattgcaaacaaatttaccatcaaacacctgtacctgtatgacgatggtagcatgaactataaagatctgtatgaacaccgcgagcaggatattaagaaactgctggcaagcagccagaatgaactggcaaagaaactggcaagccatagcaataataacgaactggatagcattagccgttatacctggcataaattctttccgaccgattatattctgctgcgtccggattatctgaccattgatgagaaaatgcagccgctgaaagaattcattggtaataatgttagcgccatgagctggtcacgttttgaaaaactgtcaccggaacagaaaaccctgtttctgaaactggttaacgtggatgaaaacaccctgcacaaactgaaaaataatagcgaagaacgcacctttatctttaccggcaccaccacctgggaaaaagacaaagataaacgtctggcaaatgcgaaaacccaggtgaaagttctggaagatttcctgaaaccggatggcaaattctatctgggcaataaaatcaaagtgttcttcaaaggtcacccgaaaggcgacgaaattaatgagtatattctgaaacagaccggtgccgaaaatattccggctaatattccgtttgaagtgctgatgatgaccaatagcctgccggattatgtaggtggtattatgagcagcatgtattttagcctgcctgccacacatattaacaaagtgatttttctggacagcgataaagtgaaaaacaagaatgatgcaaaagcacagaccctgagcaaactgatgctgatgttaaatgttattacccctgagcagatcgcctttgaggaaattccggaaaccaaaaagaacagcttctttaaacaggcctttgataccctgcgtagcaaattttaa

SEQ ID NO: 31 - DNA, 939 bp, Mannheimiasp.
  source 1..939: mol_type = other DNA
atgaacctgattatttgttgtacaccgctgcaggttctgattgcagagaaaattctggaaattcaccgcaacgaacagtttttcggtgttatgctgagcaccgttaaaaacgccaaattcgatttttatcagagccgtctggcaaagaaatgtcagcagttctttgcaatgcagcagcatagcgaacgtattcagctgctgaaagaaatcatctatctgaaaagcaccttcggtggcaaaaagttcaataaagtttttctggccaacatcaacgagctggaaatccagtttctgctgagcgcaattaactttaacgaaatcaacaccttcgatgacggcattgccaatattgttcagagcggcattttctacaaacaagaatgcagcggtattaaccgcaaactgattaatacctttctgggcaatcgttacagcctggaaaaactgaaaaagctgagcaaaaagcactataccatctataaaggcttcccgaacattatcgaaaacaccgtgtatatcgaactgatcaatagcaccacactgccggatagcgaactgaataatagcgaagttgttaatattctgctgggccagccgatttttgaacgtgatgatgagaaaaacattatcctggccgaaaaagtgattcgccagtttaacattgatcgctattttccgcatccgcgtgaaaaatatcagattagcaatgtcgagtatatcaaaaccaacctgatcctggaagattacctgtttcaagaatgtagcgataaaaagtgccgtgtgtatacctattttagcagcgcagttattaacatcctgaacaaaagcccgaatattgaagttgttgcactgcgtgttaatgtggataatccgacctatattgaaagctatgtgctgctggaaaatctgggcattaacattattgatatccgcgaataa

SEQ ID NO: 32 - DNA, 903 bp, Campylobacter subantarcticus
  source 1..903: mol_type = other DNA
atgcaaggtggtggtaatgccattatttgtggtaatggtccgagcctgaaagatatcgattataagaaactgcctcgcaagtatgatgtgtttcgttgcaatcagttctacttcgaggaaaaatactacctgggcaagaacatcaaatacgcctttttcaatccgttcgtgttcttcgaacagtattacaccaccaaaaagctgatcgagaagaaagagtataacatcgagaacattatctgcagcacctttaatctgccgaccgtggataatgaaaacttcatcaaaaacttcaacaactatttttgcgacgcctatctgggtcatgaaattctgcataacatcaaagattttctggcctttatcaaatacaacgaactgtatgaaaacaaccgtattaccagcggcatttatatgtgtgcaattgccattgcgctgggctataaaaacatttatctgtgcggcatcgatttctataacgataaaaacaacatgtacggcttcgacaacaagaaagaaaatctgctgaaactgaacccggaattcctgaaaaaggatagcgtttataccaagcacagcaaagagtttgatctgaaagcactggaatttctgaaagaaatctatggcgtgaacttctacagcctgaataataacgaactgagcaaatatatcccgctggcaccgaataccaataataactttgtgctgatcgacaaagataaaaactatgtgaacgacattctgatcccgaaagagaaagattactgcaagctgttcaaacaagaggacggtaaaatcaagctgaaagagaacgtctactataaactgttcaaagacctgtttcgtctgccgagcgatattaaacattaccttaaagagaagtacgccaacaagaaccgctaa

SEQ ID NO: 33 - DNA, 909 bp, Campylobacter coli
  source 1..909: mol_type = other DNA
atgcagaatgttattattgcaggtaatggtccgagcctgcagagcattaactatcagcgtctgccgaaagaatatgatattttccgttgcaaccagttctacttcgaggataaatactatctgggcaagaacattaaagcagccttttttaacccgtatccgtttctgcagcagtatcataccgcaaaacagctggtttttaacaacgagtacaagatcgaaaacatcttttgcagcacctttaacctgccgtttatcgagaaagacaacttcatcaacaagttctatgatttcttcccggatgcaaaactgggccataaaatcattgaaaacctgaaagagttctacgcctacatcaaatacaacgagatctatctgaacaaacgtattaccagcggcatttatatgtgtgcaattgccattgcgctgggctataaaaacatctatctgtgcggcatcgatttctatgaaggcgaaaccatttatccgtttaaagccatgagcaaaaacatcaaaaaaatctttccgtggatcaaagacttcaacccgagcaattttcacagcaaagagtatgacatcgagatcctgaaactgctggaaagcatctataaagtgaacatttatgccctgtgcgataatagcgcactggcaaactattttccgctgctggttaatacggataatagctttgttctggaaaacaaaagcgacgattgcatcaatgatattctgctgaccaataatacccctggcatcaacttctataaaagccagattcaggtgaacaacaccgaaattctgctgctgaattttcagaacatgatcagcgccaaagaaaacgaaattagcaacctgaacaaaattctgcaggacagctacaaaaccatcaacaccaaagagaacgagtaa

SEQ ID NO: 34 - DNA, 903 bp, Campylobacter jejuni
  source 1..903: mol_type = other DNA
atgacacgtacccgtatggaaaatgaactgattgtgagcaaaaacatgcagaacattatcattgcaggtaatggtccgagcctgaaaaacattaactataaacgtctgcctcgcgagtatgatgtttttcgttgtaaccagttctacttcgaggacaaatattacctgggcaaaaaaatcaaagccgtgtttttcaatccgggtgtttttctgcagcagtatcataccgcaaaacagctgattctgaaaaacgagtacgagatcaaaaacatcttttgcagcacctttaacctgccgtttattgaaagcaacgatttcctgcaccagttttacaacttttttccggatgcaaaactgggctatgaagtgattgaaaacctgaaagaattctacgcctacatcaagtacaacgagatctatttcaacaaacgcattaccagcggtgtttatatgtgtgcaattgccattgcgctgggctataaaaccatttatctgtgcggtatcgatttctatgaaggcgacgttatttatccgtttgaagcaatgagcaccaacattaaaacaatctttccgggtatcaaagacttcaaaccgagcaattgtcacagcaaagaatatgatattgaggccctgaaactgctgaaaagcatctataaagtgaacatctatgccctgtgtgatgatagcattctggcaaatcattttccgctgagcattaacatcaacaacaactttaccctggaaaacaagcacaacaacagcattaatgatatcctgctgaccgataatacaccgggtgttagcttttacaaaaatcagctgaaagccgataataagatcatgctgaacttctacaacatcctgcatagcaaagacaacctgatcaaattcctgaacaaataa

SEQ ID NO: 35 - DNA, 2818 bp, Campylobacter jejuni
  source 1..2818: mol_type = other DNA
atgaaagaaataaaaatacaaaatataatcataagtgaagaaaaagcacccttagtcgtacctgaaataggcattaatcataatggcagtttagaactagctaaaattatggtagatgcagcctttagcgcaggtgctaagattataaagcatcaaactcatattgttgaagatgagatgagtaaggccgctaaaaaagtaattcctggtaatgcaaaaataagcatttatgagattatgcaaaaatgtgctttggattataaagatgagctagcacttaaagaatacacagaaaaattaggtcttgtttatcttagcacacctttttctcgtgcaggtgcgaaccgcttagaagatatgggagttagtgcttttaagattggttcaggtgagtgtaataattatccgcttattaaacacatagcagcctttaaaaagcctatgatagttagcacaggaatgaatagtattgaaagtataaaaccaactgtaaaaatcttattagacaatgaaattccttttgttttaatgcacacgaccaatctttacccaaccccgcataatcttgtaagattaaacgctatgcttgagttaaaaaaagaattttcttgtatggtaggcttaagcgaccacacaacagataatcttgcgtgtttaggtgcagttgtacttggagcttgtgtgcttgaaagacattttactgatagtatgcatagaagtggccctgatatagtttgttctatggatacaaaggctttaaaagagctaattatacaaagtgagcaaatggctataataagaggaaataatgaaagtaaaaaagcggctaaacaagaacaagttacaattgattttgcctttgcaagtgtagttagcattaaagatattaaaaaaggcgaagttttatctatggataatatttgggttaaaagacctggacttggtggaattagtgcggctgaatttgaaaatattttaggcaaaaaagcattaagagatatagaaaatgatgctcagttaagctatgaggattttgcgtgaaaaaaatcctttttataacaggctctagggctgattattctaagattaaatctttaatgtacagggtgcaaaactcaagcgaatttgaactttacatctttgcaacaggaatgcacttaagtaaaaattttggctatacagttaaagaactttataaaaatggctttaaaaatatttatgaatttataaattatgataaatattatcaaactgataaggctttagctactacaattgatggattttcaaggtatgcaaatgagctaaaacctgatttaatcgtagtacatggagatagaattgagcctttagcagcagctattgttggagcattaaataatatcttagtagcgcatattgaaggcggagagatttcaggaactattgacgatagcttacgccacgctatatcaaaactagctcatattcatttagtaaatgatgagtttgcaaaaaggcgtttaatgcagcttggagaagatgaaaaatctatttttatcataggttcgcctgatttagaacttttaaacgataataaaatttcacttagcgaagcaaaaaaatattatgatataaattatgaaaactacgctttgcttatgtttcatcctgttacaactgaaattactagcattaaaaatcaagcagacaatttagtaaaagcactgatacaaagtaataaaaattatattgttatttatccaaataatgatttaggttttgaattaatcttgcaaagctatgaagagtttaaaaataaccctagatttaagctttttccatcgcttagatttgagtattttataactttgttaaaaaatgctgattttataataggtaattcaagttgtattttaaaagaggccttatacttaaaaacagcagggattttagttggctcaagacaaaatggaagacttggcaatgaaaatacactaaaagttaatgcaaatagtgatgaaatactaaaagctattaacactattcataaaaaacaagatttatttagcgctaagttagagattttagatagctcaaaattattttttgaatatttacaaagcggagatttttttaaactcagcacacaaaaagtttttaaggatataaaatgagcttagcaataatccctgctcgtggtggctcaaagggtattaaaaataaaaatttggttttattaaacaataaacctttaatttactacacgatcaaagctgcactaaatgctaaaagcattagtaaagttgttgtaagcagtgatagtgatgaaattttaaattatgcaaaaagtcaaaatgttgatattttaaaacgcccaattagccttgcacaagatgataccacaagcgataaagtgctgttacatgctctaaaattttataaagattatgaagatgtagtttttttacaacccacttcaccgctaagaacaaatattcatattaatgaagcttttaatctttataaaaatagcaatgcaaatgccctaattagcgtaagcgaatgtgataataaaattctaaaagcctttgtttgtaatgattgtggcgatttagcagggatttgtaatgatgaatatccttttatgccaaggcaaaaattgcctaaaacttatatgagcaatggtgcaatttatattttaaagataaaagaatttttaaacaatcctagctttttacaaagcaaaaccaagcattttttaatggacgaaagctcaagtttagatattgactgtttggaggatttaaaaaaggttgaacagatatggaaaaaataa

SEQ ID NO: 36 - protein, 332 aa, Neisseria meningitidis
MQPLVSVLICAYNVEKYFAQSLAAVVNQTWRNLEILIVDDGSTDGTLAIAKDFQKRDSRIKILAQAQNSGLIPSLNIGLDELAKSGMGEYIARTDADDIAAPDWIEKIVGEMEKDRSIIAMGAWLEVLSEEKDGNRLARHHRHGKIWKKPTRPEDIADFFPFGNPIHNNTMIMRRSVIDGGLRYNTERDWAEDYQFWYDVSKLGRLAYYPEALVKYRLHANQVSSKYSIRQHEIAQGIQKTARNDFLQSMGFKTRFDSLEYRQIKAVAYELLEKHLPEEDFERARRFLYQCFKRTDTLPAGAWLDFAADGRMRRLFTLRQYFGILHRLLKNR

SEQ ID NO: 37 - protein, 439 aa, Helicobacter pylori
MISVYIISLKESQRRLDTEKLVLESNEKFKGRCVFQIFDAISPKHEDFEKFVQELYDSSSLLKSDWFHSDYCYQELLPQEFGCYLSHYLLWKECVKLNQPVVILEDDVALESNFMQALEDCLKSPFDFVRLYGHYWGGHKTNLCALPVYTETEEAEASIEKTPIENYEVTSPPPPNPTRDTQQDFITETQQDPKELSEPCKIAPQKISFNQVVFKKIKRKLNRFIGSILARTEVYKNIVAKYDDLTTKYDDLTTKYDDLTTKYDDLTTKYDDLNKNIAEKYDELMGKYESLLAKEVNIKETFWESRADSEKEALFLDHFYLTSVYVATTAGYYLTPKGAKTFIEATERFKIIEPVDMFINNPTYHDIANFTYVPCPVSLNKHAFNSTIQNAKKPDISLKPPKKSYFDNLFYHKFNARKCLKAFNKYSKQYAPLKTPKEV

SEQ ID NO: 38 - protein, 394 aa, Rosenbergiella nectarea
MQSFTPPAPKGGNPVFMMFMLVTFFVSIAGALQAPTLSLYLSQELAAKPFMVGLFFTINAVTGIIISFILAKRSDRKGDRRRLLMFCCAMAIANALMFAFVRQYVVLITLGLILSALTSVVMPQLFALAREYADRTGREVVMFSSVMRTQMSLAWVIGPPISFALALNYGFITLYLVAAALFLLSLILIKTTLPSVPRLYPAEDLAKSAASGWKRTDVRFLFAASVLMWVCNLMYIIDMPLYISKSLGMPESFAGVLMGTAAGLEIPVMLLAGYLAKRVGKRPLVIVAAVCGLAFYPAMLVFHQQTGLLIIQLLNAVFIGIVAGLVMLWFQDLMPGKAGAATTLFTNSVSTGMIFAGLCQGLLSDLLGHQAIYVLATVLMVIALLLLLRVKEQA

SEQ ID NO: 39 - protein, 393 aa, Yersinia bercovieri
MKSALTFSRRINPVFLAFFVVAFLSGIAGALQAPTLSLFLSTEVKVRPLWVGLFYTVNAIAGITVSFILAKRSDSRGDRRKLIMVCYLMAVGNCLLFAFNRDYLTLITAGVLLASVANTAMPQIFALAREYADSSAREVVMFSSIMRAQLSLAWVIGPPLSFMLALNYGFTLMFSIAAGIFVLSALVVWFILPSVPRAEPVVDAPVVVQGSLFADKNVLLLFIASMLMWTCNTMYIIDMPLYITASLGLPERLAGLLMGTAAGLEIPIMLLAGYSVRYFGKRKIMLFAVLAGVLFYTGLVLFKFKTALMLLQIFNAIFIGIVAGIGMLYFQDLMPGRAGAATTLFTNSISTGVILAGVLQGGLTETWGHDSVYVMAMVLSILALIICARVREA

SEQ ID NO: 40 - protein, 393 aa, Yersinia frederiksenii
MKSALTFSRRINPVFLAFFVVAFLSGIAGALQAPTLSLFLSTEVKVRPLWVGLFYTVNAIAGITVSFVLAKRSDLRGDRRKLILVCYLMAVGNCLLFAFNRDYLTLITAGVLLAAVANTAMPQIFALAREYADNSAREVVMFSSIMRAQLSLAWVIGPPLSFMLALNYGFTLMFCIAAGIFVLSALVVWFILPSVQRAEPVMDAPTVAQGSLFADKDVLLLFIASMLMWTCNTMYIIDMPLYITASLGLPERLAGLLMGTAAGLEIPIMLLAGYSVRRFGKRKIMLFAVLAGVLFYTGLVLFKFKSALMLLQIFNAIFIGIVAGIGMLYFQDLMPGRAGAATTLFTNSISTGVILAGVLQGVLTETWGHNSVYVMAMILAILSLIICARVREA

SEQ ID NO: 41 - DNA, 203 bp, synthetic construct
  misc_feature 1..203: note = Promoter Sequence
  source 1..203: mol_type = other DNA
tgcgtcgccattctgtcgcaacacgccagaatgcggcggcgatcactaactcaacaaatcaggcgatgtaaccgctttcaatctgtgagtgatttcacagtatcttaacaatgtgatagctatgattgcaccgtgcctacaagcatcgtggaggtccgtgactttcacgcatacaacaaacattaaccaaaggaaaaacagct

SEQ ID NO: 42 - DNA, 203 bp, synthetic construct
  misc_feature 1..203: note = Promoter Sequence
  source 1..203: mol_type = other DNA
tgcgtcgccattctgtcgcaacacgccagaatgcggcggcgatcactaactcaacaaatcaggcgatgtaaccgctttcaatctgtgagtgatttcacagtatcttaacaatgtgatagctatgattgcaccgtgcctacaagcatcgtggaggtccgtgactttcacgcatacaacaaacattaaccaactgagaaacagct

SEQ ID NO: 43 - DNA, 203 bp, synthetic construct
  misc_feature 1..203: note = Promoter Sequence
  source 1..203: mol_type = other DNA
tgcgtcgccattctgtcgcaacacgccagaatgcggcggcgatcactaactcaacaaatcaggcgatgtaaccgctttcaatctgtgagtgatttcacagtatcttaacaatgtgatagctatgattgcaccgtgcctacaagcatcgtggaggtccgtgactttcacgcatacaacaaacattaaccaaccgagaaacagct

SEQ ID NO: 44 - DNA, 310 bp, synthetic construct
  misc_feature 1..310: note = Promoter Sequence
  source 1..310: mol_type = other DNA
atgcgcaaatgcggcacgccttgcagattacggtttgccacacttttcatccttctcctggtgacataatccacatcaatcgaaaatgttaataaatttgttgcgcgaatgatctaacaaacatgcatcatgtacaatcagatggaataaatggcgcgataacgctcattttatgacgaggcacacacattttaagttcgatatttctcgtttttgctcgttaacgataagtttacagcatgcctacaagcatcgtggaggtccgtgactttcacgcatacaacaaacattaaccaactaggaaacagct

SEQ ID NO: 45 - DNA, 203 bp, synthetic construct
  misc_feature 1..203: note = Promoter Sequence
  source 1..203: mol_type = other DNA
tgcgtcgccattctgtcgcaacacgccagaatgcggcggcgatcactaactcaacaaatcaggcgatgtaaccgctttcaatctgtgagtgatttcacagtatcttaacaatgtgatagctatgattgcaccgtgcctacaagcatcgtggaggtccgtgactttcacgcatacaacaaacattaaccaagagcaaaacagct

SEQ ID NO: 46 - DNA, 189 bp, synthetic construct
  misc_feature 1..189: note = Promoter Sequence
  source 1..189: mol_type = other DNA
gaaaacattcataaattaaatgtgaattgccgcacacattattaaataagatttacaaaatgttcaaaatgacgcatgaaatcacgtttcactttcgaattatgagcgaatatgcgcgatgcctacaagcatcgtggaggtccgtgactttcacgcatacaacaaacattaaccaaggaggaaacagct

SEQ ID NO: 47 - DNA, 239 bp, synthetic construct
  misc_feature 1..239: note = Promoter Sequence
  source 1..239: mol_type = other DNA
ccatttagccatagtaaaaacatgaattgtttgatttcgcgcatattcgctcataattcgaaagtgaaacgtgatttcatgcgtcattttgaacattttgtaaatcttatttaataatgtgtgcggcaattcacatttaatttatgaatgttttcttaacatcgcggcatgcctacaagcatcgtggaggtccgtgactttcacgcatacaacaaacattaaccaaggaggaaacagct

SEQ ID NO: 48 - DNA, 310 bp, synthetic construct
  misc_feature 1..310: note = Promoter Sequence
  source 1..310: mol_type = other DNA
atgcgcaaatgcggcacgccttgcagattacggtttgccacacttttcatccttctcctggtgacataatccacatcaatcgaaaatgttaataaatttgttgcgcgaatgatctaacaaacatgcatcatgtacaatcagatggaataaatggcgcgataacgctcattttatgacgaggcacacacattttaagttcgatatttctcgtttttgctcgttaacgataagtttacagcatgcctacaagcatcgtggaggtccgtgactttcacgcatacaacaaacattaaccaactgagaaacagct

SEQ ID NO: 49 - DNA, 310 bp, synthetic construct
  misc_feature 1..310: note = Promoter Sequence
  source 1..310: mol_type = other DNA
atgcgcaaatgcggcacgccttgcagattacggtttgccacacttttcatccttctcctggtgacataatccacatcaatcgaaaatgttaataaatttgttgcgcgaatgatctaacaaacatgcatcatgtacaatcagatggaataaatggcgcgataacgctcattttatgacgaggcacacacattttaagttcgatatttctcgtttttgctcgttaacgataagtttacagcatgcctacaagcatcgtggaggtccgtgactttcacgcatacaacaaacattaaccaaccgagaaacagct

SEQ ID NO: 50 - DNA, 310 bp, synthetic construct
  misc_feature 1..310: note = Promoter Sequence
  source 1..310: mol_type = other DNA
atgcgcaaatgcggcacgccttgcagattacggtttgccacacttttcatccttctcctggtgacataatccacatcaatcgaaaatgttaataaatttgttgcgcgaatgatctaacaaacatgcatcatgtacaatcagatggaataaatggcgcgataacgctcattttatgacgaggcacacacattttaagttcgatatttctcgtttttgctcgttaacgataagtttacagcatgcctacaagcatcgtggaggtccgtgactttcacgcatacaacaaacattaaccaagagaaaaacagct

SEQ ID NO: 51 - DNA, 350 bp, synthetic construct
  misc_feature 1..350: note = Promoter Sequence
  source 1..350: mol_type = other DNA
tgcgtcgccattctgtcgcaacacgccagaatgcggcggcgatcactaactcaacaaatcaggcgatgtaaccgctttcaatctgtgagtgatttcacagtatcttaacaatgtgatagctatgattgcaccgttttaacgttgtaacccgtatgtaacagtgaataatcacttttgccgaggtaacagcgtcataacaacaattaaagccgttttctggagcgttaccgggcatggaagaacgaattttaaaaagtgagcttcggcgttcagtaacacttcattaactctactgccccgccgagcatttatctcaagcactaccctgcataagcaaggaggaaacagct

SEQ ID NO: 52 - DNA, 310 bp, synthetic construct
  misc_feature 1..310: note = Promoter Sequence
  source 1..310: mol_type = other DNA
atgcgcaaatgcggcacgccttgcagattacggtttgccacacttttcatccttctcctggtgacataatccacatcaatcgaaaatgttaataaatttgttgcgcgaatgatctaacaaacatgcatcatgtacaatcagatggaataaatggcgcgataacgctcattttatgacgaggcacacacattttaagttcgatatttctcgtttttgctcgttaacgataagtttacagcatgcctacaagcatcgtggaggtccgtgactttcacgcatacaacaaacattaaccaaaggaaaaacagct

SEQ ID NO: 53 - DNA, 310 bp, synthetic construct
  misc_feature 1..310: note = Promoter Sequence
  source 1..310: mol_type = other DNA
atgcgcaaatgcggcacgccttgcagattacggtttgccacacttttcatccttctcctggtgacataatccacatcaatcgaaaatgttaataaatttgttgcgcgaatgatctaacaaacatgcatcatgtacaatcagatggaataaatggcgcgataacgctcattttatgacgaggcacacacattttaagttcgatatttctcgtttttgctcgttaacgataagtttacagcatgcctacaagcatcgtggaggtccgtgactttcacgcatacaacaaacattaaccaagagctaaacagct

SEQ ID NO: 54 - DNA, 189 bp, synthetic construct; identical to SEQ ID NO: 46
  misc_feature 1..189: note = Promoter Sequence
  source 1..189: mol_type = other DNA